European Patent Application EP 4 501 961 A1, published February 5, 2025. Title: MONOCLONAL ANTIBODY AGAINST HLA-G1, -G2, -G5 AND HLA-G6 ISOFORMS AND USE THEREOF. Applicant: TAIZHOU ENZE MEDICAL CENTER (GROUP). The sequence listing filed with the application follows.

SEQUENCE LISTING (19 sequences)

SEQ ID NO: 1 - protein, 112 aa, (Hybridoma)（YWHG-3)
DIMMTQTPLSLPVSLGDQASISCRSSQSLVHSTGNTFLNWYLQKPGQSPKLLIYKVSNRFSGVSDRFSGSGSGTDFTLKIRRVEAEDLGVYFCSQSTHVPWTFGGGTKLEIK

SEQ ID NO: 2 - protein, 11 aa, (Hybridoma)（YWHG-3)
QSLVHSTGNTF

SEQ ID NO: 3 - protein, 3 aa, (Hybridoma)（YWHG-3)
KVS

SEQ ID NO: 4 - protein, 9 aa, (Hybridoma)（YWHG-3)
SQSTHVPWT

SEQ ID NO: 5 - protein, 112 aa, (Hybridoma)（YWHG-3)
LVQLQQSGGGLVKPGGSLKLSCAASGFTFSDYNMYWVRQTPEKRLEWVATISDGGRSTFYLDSVKGRFTISRDNAKNNLYLQINNLKSEDTAIYYCVRDDYWGQGTTLTVSS

SEQ ID NO: 6 - protein, 8 aa, (Hybridoma)（YWHG-3)
GFTFSDYN

SEQ ID NO: 7 - protein, 8 aa, (Hybridoma)（YWHG-3)
ISDGGRST

SEQ ID NO: 8 - protein, 5 aa, (Hybridoma)（YWHG-3)
VRDDY

SEQ ID NO: 9 - protein, 26 aa, (Hybridoma)（YWHG-3)
DIMMTQTPLSLPVSLGDQASISCRSS

SEQ ID NO: 10 - protein, 17 aa, (Hybridoma)（YWHG-3)
LNWYLQKPGQSPKLLIY

SEQ ID NO: 11 - protein, 36 aa, (Hybridoma)（YWHG-3)
NRFSGVSDRFSGSGSGTDFTLKIRRVEAEDLGVYFC

SEQ ID NO: 12 - protein, 10 aa, (Hybridoma)（YWHG-3)
FGGGTKLEIK

SEQ ID NO: 13 - protein, 25 aa, (Hybridoma)（YWHG-3)
LVQLQQSGGGLVKPGGSLKLSCAAS

SEQ ID NO: 14 - protein, 17 aa, (Hybridoma)（YWHG-3)
MYWVRQTPEKRLEWVAT

SEQ ID NO: 15 - protein, 38 aa, (Hybridoma)（YWHG-3)
FYLDSVKGRFTISRDNAKNNLYLQINNLKSEDTAIYYC

SEQ ID NO: 16 - protein, 11 aa, (Hybridoma)（YWHG-3)
WGQGTTLTVSS

SEQ ID NO: 17 - DNA, 334 bp, (Hybridoma)（YWHG-3)
gatatcatgatgacccaaactccactctccctgcctgtcagtcttggagatcaagcctccatctcttgcagatctagtcagagccttgtacacagtactggaaacacctttttaaattggtacctgcgaagccaggccagtctccaaagctcctgatctacaaagtttccaaccgattttctggggtctcagacaggttcagtggcagtggatcagggacagatttcacactcaagatccgcagagtggaggctaagatctgggagtttatttctgctctcaaagtacacatgttccgtggacgttcggtggaggcaccaagctggaaatcaaa

SEQ ID NO: 18 - DNA, 334 bp, (Hybridoma)（YWHG-3)
ttagtgcagctgcagcagtcagggggaggcttagtgaagcctggagggtccctgaaactctcctgtgcagcctctggattcaccttcagtgactataatatgtattgggttcgccagactccggaaagaggctggagtgggtcgcaaccattagtgatggtggtcgttccaccttctatctagacagtgtgaaggggcgattcaccatctccagagacaatgccaagaacaacctatacctgcagatcaacaattgaagtctgaggacacagccatatattactgtgtaagagatgactattggggccaaggcaccactctcacagtctcctca

SEQ ID NO: 19 - protein, 18 aa, 2 Ambystoma laterale x Ambystoma jeffersonianum
KTHVTHHPVFDYEATLRC